European Patent Specification EP 4 208 213 B1, published June 10, 2026. Title: METHOD FOR PRODUCING MACROPOROUS SCAFFOLDS COMPOSED OF SILK AND CALCIUM PHOSPHATE. Applicant: Spiber Technologies AB. The sequence listing filed with the application follows.

SEQUENCE LISTING (17 sequences)

SEQ ID NO: 1 - protein, 263 aa, Euprosthenops australis
  DOMAIN (1)..(158): REP fragment
  DOMAIN (159)..(165): Spacer fragment
  DOMAIN (166)..(263): CT fragment
GPNSGQGGYGGLGQGGYGQGAGSSAAAAAAAAAAAAGGQGGQGQGGYGQGSGGSAAAAAAAAAAAAAAAGRGQGGYGQGSGGNAAAAAAAAAAAAAAAGQGGQGGYGRQSQGAGSAAAAAAAAAAAAAAGSGQGGYGGQGQGGYGQSSASASAAASAASTVANSVSRLSSPSAVSRVSSAVSSLVSNGQVNMAALPNIISNISSSVSASAPGASGCEVIVQALLEVITALVQIVSSSSVGYINPSAVNQITNVVANAMAQVMG

SEQ ID NO: 2 - protein, 339 aa, Artificial Sequence
  Fusion protein
MGSSGHHHHHHMVDNKFNKEQQNAFYEILHLPNLNEEQRNAFIQSLKDDPSQSANLLAEAKKLNDAQAPKLEALFQGPNSGQGGYGGLGQGGYGQGAGSSAAAAAAAAAAAAGGQGGQGQGGYGQGSGGSAAAAAAAAAAAAAAAGRGQGGYGQGSGGNAAAAAAAAAAAAAAAGQGGQGGYGRQSQGAGSAAAAAAAAAAAAAAGSGQGGYGGQGQGGYGQSSASASAAASAASTVANSVSRLSSPSAVSRVSSAVSSLVSNGQVNMAALPNIISNISSSVSASAPGASGCEVIVQALLEVITALVQIVSSSSVGYINPSAVNQITNVVANAMAQVMG

SEQ ID NO: 3 - protein, 276 aa, Artificial Sequence
  Fusion protein
  DISULFID (5)..(14)
GPNSCTGRGDSPACPNSGQGGYGGLGQGGYGQGAGSSAAAAAAAAAAAAGGQGGQGQGGYGQGSGGSAAAAAAAAAAAAAAAGRGQGGYGQGSGGNAAAAAAAAAAAAAAAGQGGQGGYGRQSQGAGSAAAAAAAAAAAAAAGSGQGGYGGQGQGGYGQSSASASAAASAASTVANSVSRLSSPSAVSRVSSAVSSLVSNGQVNMAALPNIISNISSSVSASAPGASGCEVIVQALLEVITALVQIVSSSSVGYINPSAVNQITNVVANAMAQVMG

SEQ ID NO: 4 - protein, 98 aa, Euprosthenops australis
SRLSSPSAVSRVSSAVSSLVSNGQVNMAALPNIISNISSSVSASAPGASGCEVIVQALLEVITALVQIVSSSSVGYINPSAVNQITNVVANAMAQVMG

SEQ ID NO: 5 - protein, 93 aa, Araneus ventricosus
NRLSSAEAASRVSSNIAAIASGGASALPSVISNIYSGVVASGVSSNEALIQALLELLSALVHVLSSASIGNVSSVGVDSTLNVVQDSVGQYVG

SEQ ID NO: 6 - protein, 5 aa, Homo sapiens
IKVAV

SEQ ID NO: 7 - protein, 5 aa, Homo sapiens
YIGSR

SEQ ID NO: 8 - protein, 5 aa, Homo sapiens
EPDIM

SEQ ID NO: 9 - protein, 5 aa, Homo sapiens
NKDIL

SEQ ID NO: 10 - protein, 5 aa, Homo sapiens
GRKRK

SEQ ID NO: 11 - protein, 15 aa, Homo sapiens
KYGAASIKVAVSADR

SEQ ID NO: 12 - protein, 12 aa, Homo sapiens
NGEPRGDTYRAY

SEQ ID NO: 13 - protein, 11 aa, Homo sapiens
PQVTRGDVFTM

SEQ ID NO: 14 - protein, 12 aa, Homo sapiens
AVTGRGDSPASS

SEQ ID NO: 15 - protein, 8 aa, Homo sapiens
TGRGDSPA

SEQ ID NO: 16 - protein, 10 aa, Artificial Sequence
  Modified from Homo sapiens
  DISULFID (1)..(10)
CTGRGDSPAC

SEQ ID NO: 17 - protein, 10 aa, Artificial Sequence
  cell-binding peptide
  misc_feature: X = any amino acid other than Cys
  DISULFID (1)..(10)
CXXRGDXXXC